European Patent Specification EP 3 897 695 B1, published June 25, 2025. Title: RECOMBINANT VECTORS FOR THE LONG TERM TREATMENT OF MUCCHOPOLYSACHARIDOSIS. Applicant: Esteve Pharmaceuticals, S.A. Universidad Autónoma de Barcelona. The sequence listing filed with the application follows.

SEQUENCE LISTING (2 sequences)

SEQ ID NO: 1 - DNA, 1515 bp, Artificial Sequence
  optimized sequence of the human sulfamidase gene sequence
gccaccatgagctgccctgtgcccgcctgttgtgccctgctgctggtgctgggactgtgcagagccagaccccggaacgctctgctgctgctggccgacgatggcggatttgagagcggcgcctacaacaacagcgccattgccacccctcatctggacgccctggccagaagaagcctgctgttccggaacgccttcaccagcgtgtccagctgcagccctagcagagcttccctgctgacaggcctgccccagcatcagaatggcatgtacggcctgcaccaggatgtgcatcacttcaacagcttcgacaaagtgcggagcctgccactgctcctgtcacaggctggcgtgagaaccggcatcatcggcaagaaacacgtgggccccgagacagtgtaccccttcgacttcgcctacaccgaagagaacggcagcgtgctgcaggtcggccggaacatcacccggatcaagctgctcgtgcggaagtttctccagacccaggacgaccggcccttcttcctgtacgtggccttccacgaccctcacagatgcggccacagccagccccagtacggcaccttctgcgagaagttcggcaacggcgagagcggcatgggcagaatccccgactggaccccccaggcatacgaccctctggacgtgctggtgccctacttcgtgcccaacacccctgccgccagagctgatctggccgcccagtacaccaccgtgggcagaatggatcagggcgtgggcctggtgctgcaggaactgagggacgctggcgtgctgaacgacaccctggtcatcttcacctccgacaacggcatcccattccccagcggccggaccaatctgtactggcccggcacagccgaacctctgctggtgtccagccccgagcaccctaagagatggggccaggtgtccgaggcctacgtgtccctgctggacctgacccccaccatcctggactggttcagcatcccctaccccagctacgccatctttggaagcaagaccatccacctgaccggcagatctctgctgcctgccctggaagctgagcctctgtgggccaccgtgttcggcagccagagccaccacgaagtgaccatgagctaccccatgcggagcgtgcagcaccggcacttccggctggtgcacaacctgaacttcaagatgcccttcccaatcgaccaggacttttacgtgtcccccaccttccaggacctgctgaacagaaccacagccggccagcccaccggctggtacaaggacctgcggcactactactaccgggccagatgggagctgtacgacagaagccgggacccccacgagacacagaacctggccaccgaccccagattcgcccagctcctggaaatgctgcgggaccagctggccaagtggcagtgggagacacacgacccttgggtctgcgctcccgacggcgtgctggaagagaagctgtccccccagtgccagccactgcacaacgagctgtga

SEQ ID NO: 2 - protein, 502 aa, Homo sapiens
MSCPVPACCALLLVLGLCRARPRNALLLLADDGGFESGAYNNSAIATPHLDALARRSLLFRNAFTSVSSCSPSRASLLTGLPQHQNGMYGLHQDVHHFNSFDKVRSLPLLLSQAGVRTGIIGKKHVGPETVYPFDFAYTEENGSVLQVGRNITRIKLLVRKFLQTQDDRPFFLYVAFHDPHRCGHSQPQYGTFCEKFGNGESGMGRIPDWTPQAYDPLDVLVPYFVPNTPAARADLAAQYTTVGRMDQGVGLVLQELRDAGVLNDTLVIFTSDNGIPFPSGRTNLYWPGTAEPLLVSSPEHPKRWGQVSEAYVSLLDLTPTILDWFSIPYPSYAIFGSKTIHLTGRSLLPALEAEPLWATVFGSQSHHEVTMSYPMRSVQHRHFRLVHNLNFKMPFPIDQDFYVSPTFQDLLNRTTAGQPTGWYKDLRHYYYRARWELYDRSRDPHETQNLATDPRFAQLLEMLRDQLAKWQWETHDPWVCAPDGVLEEKLSPQCQPLHNEL